European Patent Specification EP 3 452 614 B1, published June 28, 2023. Title: ACCURATE MOLECULAR BARCODING. Applicant: Eleen Shum, et al. The sequence listing filed with the application follows.

SEQUENCE LISTING (97 sequences)

SEQ ID NO: 1 - DNA, 49 bp, Artificial Sequence
  Synthetic nucleotide
  misc_feature (29)..(36): n is a, c, g, or t
acacgacgctcttccgatctacagtgctnnnnnnnncagacagacttgt

SEQ ID NO: 2 - DNA, 49 bp, Artificial Sequence
  Synthetic nucleotide
  misc_feature (29)..(36): n is a, c, g, or t
acacgacgctcttccgatctacatgcgtnnnnnnnncagacagacttgt

SEQ ID NO: 3 - DNA, 49 bp, Artificial Sequence
  Synthetic nucleotide
  misc_feature (29)..(36): n is a, c, g, or t
acacgacgctcttccgatctaccgattgnnnnnnnncagacagacttgt

SEQ ID NO: 4 - DNA, 49 bp, Artificial Sequence
  Synthetic nucleotide
  misc_feature (29)..(36): n is a, c, g, or t
acacgacgctcttccgatctaccttgagnnnnnnnncagacagacttgt

SEQ ID NO: 5 - DNA, 49 bp, Artificial Sequence
  Synthetic nucleotide
  misc_feature (29)..(36): n is a, c, g, or t
acacgacgctcttccgatctacgatgtcnnnnnnnncagacagacttgt

SEQ ID NO: 6 - DNA, 49 bp, Artificial Sequence
  Synthetic nucleotide
  misc_feature (29)..(36): n is a, c, g, or t
acacgacgctcttccgatctacgtatgcnnnnnnnncagacagacttgt

SEQ ID NO: 7 - DNA, 49 bp, Artificial Sequence
  Synthetic nucleotide
  misc_feature (29)..(36): n is a, c, g, or t
acacgacgctcttccgatctactctggannnnnnnncagacagacttgt

SEQ ID NO: 8 - DNA, 49 bp, Artificial Sequence
  Synthetic nucleotide
  misc_feature (29)..(36): n is a, c, g, or t
acacgacgctcttccgatctactggctannnnnnnncagacagacttgt

SEQ ID NO: 9 - DNA, 49 bp, Artificial Sequence
  Synthetic nucleotide
  misc_feature (29)..(36): n is a, c, g, or t
acacgacgctcttccgatctagaccttgnnnnnnnncagacagacttgt

SEQ ID NO: 10 - DNA, 49 bp, Artificial Sequence
  Synthetic nucleotide
  misc_feature (29)..(36): n is a, c, g, or t
acacgacgctcttccgatctagattccgnnnnnnnncagacagacttgt

SEQ ID NO: 11 - DNA, 49 bp, Artificial Sequence
  Synthetic nucleotide
  misc_feature (29)..(36): n is a, c, g, or t
acacgacgctcttccgatctagccgaccnnnnnnnncagacagacttgt

SEQ ID NO: 12 - DNA, 49 bp, Artificial Sequence
  Synthetic nucleotide
  misc_feature (29)..(36): n is a, c, g, or t
acacgacgctcttccgatctagcgctgcnnnnnnnncagacagacttgt

SEQ ID NO: 13 - DNA, 52 bp, Artificial Sequence
  Synthetic nucleotide
  misc_feature (29)..(36): n is a, c, g, or t
acacgacgctcttccgatctagctagtcnnnnnnnntttcagacagacttgt

SEQ ID NO: 14 - DNA, 52 bp, Artificial Sequence
  Synthetic nucleotide
  misc_feature (29)..(36): n is a, c, g, or t
acacgacgctcttccgatctaggctctannnnnnnntttcagacagacttgt

SEQ ID NO: 15 - DNA, 52 bp, Artificial Sequence
  Synthetic nucleotide
  misc_feature (29)..(36): n is a, c, g, or t
acacgacgctcttccgatctaggtctcannnnnnnntttcagacagacttgt

SEQ ID NO: 16 - DNA, 52 bp, Artificial Sequence
  Synthetic nucleotide
  misc_feature (29)..(36): n is a, c, g, or t
acacgacgctcttccgatctagtactatnnnnnnnntttcagacagacttgt

SEQ ID NO: 17 - DNA, 52 bp, Artificial Sequence
  Synthetic nucleotide
  misc_feature (29)..(36): n is a, c, g, or t
acacgacgctcttccgatctagtcagctnnnnnnnntttcagacagacttgt

SEQ ID NO: 18 - DNA, 52 bp, Artificial Sequence
  Synthetic nucleotide
  misc_feature (29)..(36): n is a, c, g, or t
acacgacgctcttccgatctagtgtcgtnnnnnnnntttcagacagacttgt

SEQ ID NO: 19 - DNA, 52 bp, Artificial Sequence
  Synthetic nucleotide
  misc_feature (29)..(36): n is a, c, g, or t
acacgacgctcttccgatctatacgtgcnnnnnnnntttcagacagacttgt

SEQ ID NO: 20 - DNA, 52 bp, Artificial Sequence
  Synthetic nucleotide
  misc_feature (29)..(36): n is a, c, g, or t
acacgacgctcttccgatctatagcgtcnnnnnnnntttcagacagacttgt

SEQ ID NO: 21 - DNA, 52 bp, Artificial Sequence
  Synthetic nucleotide
  misc_feature (29)..(36): n is a, c, g, or t
acacgacgctcttccgatctatcggtcannnnnnnntttcagacagacttgt

SEQ ID NO: 22 - DNA, 52 bp, Artificial Sequence
  Synthetic nucleotide
  misc_feature (29)..(36): n is a, c, g, or t
acacgacgctcttccgatctatctcggannnnnnnntttcagacagacttgt

SEQ ID NO: 23 - DNA, 52 bp, Artificial Sequence
  Synthetic nucleotide
  misc_feature (29)..(36): n is a, c, g, or t
acacgacgctcttccgatctatgacgctnnnnnnnntttcagacagacttgt

SEQ ID NO: 24 - DNA, 52 bp, Artificial Sequence
  Synthetic nucleotide
  misc_feature (29)..(36): n is a, c, g, or t
acacgacgctcttccgatctattccgagnnnnnnnntttcagacagacttgt

SEQ ID NO: 25 - DNA, 54 bp, Artificial Sequence
  Synthetic nucleotide
  misc_feature (29)..(36): n is a, c, g, or t
acacgacgctcttccgatctattgaccgnnnnnnnntttttcagacagacttgt

SEQ ID NO: 26 - DNA, 54 bp, Artificial Sequence
  Synthetic nucleotide
  misc_feature (29)..(36): n is a, c, g, or t
acacgacgctcttccgatctcagagttcnnnnnnnntttttcagacagacttgt

SEQ ID NO: 27 - DNA, 54 bp, Artificial Sequence
  Synthetic nucleotide
  misc_feature (29)..(36): n is a, c, g, or t
acacgacgctcttccgatctcagccgacnnnnnnnntttttcagacagacttgt

SEQ ID NO: 28 - DNA, 54 bp, Artificial Sequence
  Synthetic nucleotide
  misc_feature (29)..(36): n is a, c, g, or t
acacgacgctcttccgatctcagttagcnnnnnnnntttttcagacagacttgt

SEQ ID NO: 29 - DNA, 54 bp, Artificial Sequence
  Synthetic nucleotide
  misc_feature (29)..(36): n is a, c, g, or t
acacgacgctcttccgatctcatcgtgannnnnnnntttttcagacagacttgt

SEQ ID NO: 30 - DNA, 54 bp, Artificial Sequence
  Synthetic nucleotide
  misc_feature (29)..(36): n is a, c, g, or t
acacgacgctcttccgatctcatgcgtannnnnnnntttttcagacagacttgt

SEQ ID NO: 31 - DNA, 54 bp, Artificial Sequence
  Synthetic nucleotide
  misc_feature (29)..(36): n is a, c, g, or t
acacgacgctcttccgatctccagttagnnnnnnnntttttcagacagacttgt

SEQ ID NO: 32 - DNA, 54 bp, Artificial Sequence
  Synthetic nucleotide
  misc_feature (29)..(36): n is a, c, g, or t
acacgacgctcttccgatctccatggcgnnnnnnnntttttcagacagacttgt

SEQ ID NO: 33 - DNA, 54 bp, Artificial Sequence
  Synthetic nucleotide
  misc_feature (29)..(36): n is a, c, g, or t
acacgacgctcttccgatctccgattgannnnnnnntttttcagacagacttgt

SEQ ID NO: 34 - DNA, 54 bp, Artificial Sequence
  Synthetic nucleotide
  misc_feature (29)..(36): n is a, c, g, or t
acacgacgctcttccgatctcgaccagcnnnnnnnntttttcagacagacttgt

SEQ ID NO: 35 - DNA, 54 bp, Artificial Sequence
  Synthetic nucleotide
  misc_feature (29)..(36): n is a, c, g, or t
acacgacgctcttccgatctcgagattcnnnnnnnntttttcagacagacttgt

SEQ ID NO: 36 - DNA, 54 bp, Artificial Sequence
  Synthetic nucleotide
  misc_feature (29)..(36): n is a, c, g, or t
acacgacgctcttccgatctcgattgacnnnnnnnntttttcagacagacttgt

SEQ ID NO: 37 - DNA, 49 bp, Artificial Sequence
  Synthetic nucleotide
  misc_feature (21)..(28): n is a, c, g, or t
acacgacgctcttccgatctnnnnnnnncgcatgtacagacagacttgt

SEQ ID NO: 38 - DNA, 49 bp, Artificial Sequence
  Synthetic nucleotide
  misc_feature (21)..(28): n is a, c, g, or t
acacgacgctcttccgatctnnnnnnnncgctatgacagacagacttgt

SEQ ID NO: 39 - DNA, 49 bp, Artificial Sequence
  Synthetic nucleotide
  misc_feature (21)..(28): n is a, c, g, or t
acacgacgctcttccgatctnnnnnnnncgtacatgcagacagacttgt

SEQ ID NO: 40 - DNA, 49 bp, Artificial Sequence
  Synthetic nucleotide
  misc_feature (21)..(28): n is a, c, g, or t
acacgacgctcttccgatctnnnnnnnncgtcatagcagacagacttgt

SEQ ID NO: 41 - DNA, 49 bp, Artificial Sequence
  Synthetic nucleotide
  misc_feature (21)..(28): n is a, c, g, or t
acacgacgctcttccgatctnnnnnnnnctacgacacagacagacttgt

SEQ ID NO: 42 - DNA, 49 bp, Artificial Sequence
  Synthetic nucleotide
  misc_feature (21)..(28): n is a, c, g, or t
acacgacgctcttccgatctnnnnnnnnctagctgacagacagacttgt

SEQ ID NO: 43 - DNA, 49 bp, Artificial Sequence
  Synthetic nucleotide
  misc_feature (21)..(28): n is a, c, g, or t
acacgacgctcttccgatctnnnnnnnnctatagtacagacagacttgt

SEQ ID NO: 44 - DNA, 49 bp, Artificial Sequence
  Synthetic nucleotide
  misc_feature (21)..(28): n is a, c, g, or t
acacgacgctcttccgatctnnnnnnnnctgactagcagacagacttgt

SEQ ID NO: 45 - DNA, 49 bp, Artificial Sequence
  Synthetic nucleotide
  misc_feature (21)..(28): n is a, c, g, or t
acacgacgctcttccgatctnnnnnnnnctgcagcgcagacagacttgt

SEQ ID NO: 46 - DNA, 49 bp, Artificial Sequence
  Synthetic nucleotide
  misc_feature (21)..(28): n is a, c, g, or t
acacgacgctcttccgatctnnnnnnnnctgtgatgcagacagacttgt

SEQ ID NO: 47 - DNA, 49 bp, Artificial Sequence
  Synthetic nucleotide
  misc_feature (21)..(28): n is a, c, g, or t
acacgacgctcttccgatctnnnnnnnncttagagccagacagacttgt

SEQ ID NO: 48 - DNA, 49 bp, Artificial Sequence
  Synthetic nucleotide
  misc_feature (21)..(28): n is a, c, g, or t
acacgacgctcttccgatctnnnnnnnncttgagaccagacagacttgt

SEQ ID NO: 49 - DNA, 52 bp, Artificial Sequence
  Synthetic nucleotide
  misc_feature (21)..(28): n is a, c, g, or t
acacgacgctcttccgatctnnnnnnnngaccagcctttcagacagacttgt

SEQ ID NO: 50 - DNA, 52 bp, Artificial Sequence
  Synthetic nucleotide
  misc_feature (21)..(28): n is a, c, g, or t
acacgacgctcttccgatctnnnnnnnngacgtcgctttcagacagacttgt

SEQ ID NO: 51 - DNA, 52 bp, Artificial Sequence
  Synthetic nucleotide
  misc_feature (21)..(28): n is a, c, g, or t
acacgacgctcttccgatctnnnnnnnngactgatctttcagacagacttgt

SEQ ID NO: 52 - DNA, 52 bp, Artificial Sequence
  Synthetic nucleotide
  misc_feature (21)..(28): n is a, c, g, or t
acacgacgctcttccgatctnnnnnnnngagccttatttcagacagacttgt

SEQ ID NO: 53 - DNA, 52 bp, Artificial Sequence
  Synthetic nucleotide
  misc_feature (21)..(28): n is a, c, g, or t
acacgacgctcttccgatctnnnnnnnngagttccatttcagacagacttgt

SEQ ID NO: 54 - DNA, 52 bp, Artificial Sequence
  Synthetic nucleotide
  misc_feature (21)..(28): n is a, c, g, or t
acacgacgctcttccgatctnnnnnnnngatatcattttcagacagacttgt

SEQ ID NO: 55 - DNA, 52 bp, Artificial Sequence
  Synthetic nucleotide
  misc_feature (21)..(28): n is a, c, g, or t
acacgacgctcttccgatctnnnnnnnngatcgacttttcagacagacttgt

SEQ ID NO: 56 - DNA, 52 bp, Artificial Sequence
  Synthetic nucleotide
  misc_feature (21)..(28): n is a, c, g, or t
acacgacgctcttccgatctnnnnnnnngatgctgttttcagacagacttgt

SEQ ID NO: 57 - DNA, 52 bp, Artificial Sequence
  Synthetic nucleotide
  misc_feature (21)..(28): n is a, c, g, or t
acacgacgctcttccgatctnnnnnnnngcagtatctttcagacagacttgt

SEQ ID NO: 58 - DNA, 52 bp, Artificial Sequence
  Synthetic nucleotide
  misc_feature (21)..(28): n is a, c, g, or t
acacgacgctcttccgatctnnnnnnnngcatgtactttcagacagacttgt

SEQ ID NO: 59 - DNA, 52 bp, Artificial Sequence
  Synthetic nucleotide
  misc_feature (21)..(28): n is a, c, g, or t
acacgacgctcttccgatctnnnnnnnngccagttatttcagacagacttgt

SEQ ID NO: 60 - DNA, 52 bp, Artificial Sequence
  Synthetic nucleotide
  misc_feature (21)..(28): n is a, c, g, or t
acacgacgctcttccgatctnnnnnnnngccgaccatttcagacagacttgt

SEQ ID NO: 61 - DNA, 54 bp, Artificial Sequence
  Synthetic nucleotide
  misc_feature (21)..(28): n is a, c, g, or t
acacgacgctcttccgatctnnnnnnnngccttagatttttcagacagacttgt

SEQ ID NO: 62 - DNA, 54 bp, Artificial Sequence
  Synthetic nucleotide
  misc_feature (21)..(28): n is a, c, g, or t
acacgacgctcttccgatctnnnnnnnngcgatacttttttcagacagacttgt

SEQ ID NO: 63 - DNA, 54 bp, Artificial Sequence
  Synthetic nucleotide
  misc_feature (21)..(28): n is a, c, g, or t
acacgacgctcttccgatctnnnnnnnngcgtacattttttcagacagacttgt

SEQ ID NO: 64 - DNA, 54 bp, Artificial Sequence
  Synthetic nucleotide
  misc_feature (21)..(28): n is a, c, g, or t
acacgacgctcttccgatctnnnnnnnnggcattgttttttcagacagacttgt

SEQ ID NO: 65 - DNA, 54 bp, Artificial Sequence
  Synthetic nucleotide
  misc_feature (21)..(28): n is a, c, g, or t
acacgacgctcttccgatctnnnnnnnnggcgccattttttcagacagacttgt

SEQ ID NO: 66 - DNA, 54 bp, Artificial Sequence
  Synthetic nucleotide
  misc_feature (21)..(28): n is a, c, g, or t
acacgacgctcttccgatctnnnnnnnnggtgttactttttcagacagacttgt

SEQ ID NO: 67 - DNA, 54 bp, Artificial Sequence
  Synthetic nucleotide
  misc_feature (21)..(28): n is a, c, g, or t
acacgacgctcttccgatctnnnnnnnngtacgcattttttcagacagacttgt

SEQ ID NO: 68 - DNA, 54 bp, Artificial Sequence
  Synthetic nucleotide
  misc_feature (21)..(28): n is a, c, g, or t
acacgacgctcttccgatctnnnnnnnngtcggctgtttttcagacagacttgt

SEQ ID NO: 69 - DNA, 54 bp, Artificial Sequence
  Synthetic nucleotide
  misc_feature (21)..(28): n is a, c, g, or t
acacgacgctcttccgatctnnnnnnnngtgacatctttttcagacagacttgt

SEQ ID NO: 70 - DNA, 54 bp, Artificial Sequence
  Synthetic nucleotide
  misc_feature (21)..(28): n is a, c, g, or t
acacgacgctcttccgatctnnnnnnnngtgcatactttttcagacagacttgt

SEQ ID NO: 71 - DNA, 54 bp, Artificial Sequence
  Synthetic nucleotide
  misc_feature (21)..(28): n is a, c, g, or t
acacgacgctcttccgatctnnnnnnnngtgtgcgctttttcagacagacttgt

SEQ ID NO: 72 - DNA, 54 bp, Artificial Sequence
  Synthetic nucleotide
  misc_feature (21)..(28): n is a, c, g, or t
acacgacgctcttccgatctnnnnnnnngttagccatttttcagacagacttgt

SEQ ID NO: 73 - DNA, 49 bp, Artificial Sequence
  Synthetic nucleotide
  misc_feature (29)..(36): h is a, c, or t
acacgacgctcttccgatctgttccagahhhhhhhhcagacagacttgt

SEQ ID NO: 74 - DNA, 49 bp, Artificial Sequence
  Synthetic nucleotide
  misc_feature (29)..(36): h is a, c, or t
acacgacgctcttccgatcttacgtgcahhhhhhhhcagacagacttgt

SEQ ID NO: 75 - DNA, 49 bp, Artificial Sequence
  Synthetic nucleotide
  misc_feature (29)..(36): h is a, c, or t
acacgacgctcttccgatcttactgcgahhhhhhhhcagacagacttgt

SEQ ID NO: 76 - DNA, 49 bp, Artificial Sequence
  Synthetic nucleotide
  misc_feature (29)..(36): h is a, c, or t
acacgacgctcttccgatcttagagccthhhhhhhhcagacagacttgt

SEQ ID NO: 77 - DNA, 49 bp, Artificial Sequence
  Synthetic nucleotide
  misc_feature (29)..(36): h is a, c, or t
acacgacgctcttccgatcttagccagthhhhhhhhcagacagacttgt

SEQ ID NO: 78 - DNA, 49 bp, Artificial Sequence
  Synthetic nucleotide
  misc_feature (29)..(36): h is a, c, or t
acacgacgctcttccgatcttatcgcaghhhhhhhhcagacagacttgt

SEQ ID NO: 79 - DNA, 49 bp, Artificial Sequence
  Synthetic nucleotide
  misc_feature (29)..(36): h is a, c, or t
acacgacgctcttccgatcttcagtcgahhhhhhhhcagacagacttgt

SEQ ID NO: 80 - DNA, 49 bp, Artificial Sequence
  Synthetic nucleotide
  misc_feature (29)..(36): h is a, c, or t
acacgacgctcttccgatcttcatgatahhhhhhhhcagacagacttgt

SEQ ID NO: 81 - DNA, 49 bp, Artificial Sequence
  Synthetic nucleotide
  misc_feature (29)..(36): h is a, c, or t
acacgacgctcttccgatcttccagagthhhhhhhhcagacagacttgt

SEQ ID NO: 82 - DNA, 49 bp, Artificial Sequence
  Synthetic nucleotide
  misc_feature (29)..(36): h is a, c, or t
acacgacgctcttccgatcttccgagathhhhhhhhcagacagacttgt

SEQ ID NO: 83 - DNA, 49 bp, Artificial Sequence
  Synthetic nucleotide
  misc_feature (29)..(36): h is a, c, or t
acacgacgctcttccgatcttcgatcaghhhhhhhhcagacagacttgt

SEQ ID NO: 84 - DNA, 49 bp, Artificial Sequence
  Synthetic nucleotide
  misc_feature (29)..(36): h is a, c, or t
acacgacgctcttccgatcttcgcgacghhhhhhhhcagacagacttgt

SEQ ID NO: 85 - DNA, 49 bp, Artificial Sequence
  Synthetic nucleotide
  misc_feature (29)..(29): h is a, c, or t
  misc_feature (30)..(30): n is a, c, g, or t
  misc_feature (31)..(31): h is a, c, or t
  misc_feature (32)..(32): n is a, c, g, or t
  misc_feature (33)..(33): h is a, c, or t
  misc_feature (34)..(34): n is a, c, g, or t
  misc_feature (35)..(35): h is a, c, or t
  misc_feature (36)..(36): n is a, c, g, or t
acacgacgctcttccgatcttcggctgghnhnhnhncagacagacttgt

SEQ ID NO: 86 - DNA, 49 bp, Artificial Sequence
  Synthetic nucleotide
  misc_feature (29)..(29): h is a, c, or t
  misc_feature (30)..(30): n is a, c, g, or t
  misc_feature (31)..(31): h is a, c, or t
  misc_feature (32)..(32): n is a, c, g, or t
  misc_feature (33)..(33): h is a, c, or t
  misc_feature (34)..(34): n is a, c, g, or t
  misc_feature (35)..(35): h is a, c, or t
  misc_feature (36)..(36): n is a, c, g, or t
acacgacgctcttccgatcttcgtagtghnhnhnhncagacagacttgt

SEQ ID NO: 87 - DNA, 49 bp, Artificial Sequence
  Synthetic nucleotide
  misc_feature (29)..(29): h is a, c, or t
  misc_feature (30)..(30): n is a, c, g, or t
  misc_feature (31)..(31): h is a, c, or t
  misc_feature (32)..(32): n is a, c, g, or t
  misc_feature (33)..(33): h is a, c, or t
  misc_feature (34)..(34): n is a, c, g, or t
  misc_feature (35)..(35): h is a, c, or t
  misc_feature (36)..(36): n is a, c, g, or t
acacgacgctcttccgatcttgaccgathnhnhnhncagacagacttgt

SEQ ID NO: 88 - DNA, 49 bp, Artificial Sequence
  Synthetic nucleotide
  misc_feature (29)..(29): h is a, c, or t
  misc_feature (30)..(30): n is a, c, g, or t
  misc_feature (31)..(31): h is a, c, or t
  misc_feature (32)..(32): n is a, c, g, or t
  misc_feature (33)..(33): h is a, c, or t
  misc_feature (34)..(34): n is a, c, g, or t
  misc_feature (35)..(35): h is a, c, or t
  misc_feature (36)..(36): n is a, c, g, or t
acacgacgctcttccgatcttgagaccthnhnhnhncagacagacttgt

SEQ ID NO: 89 - DNA, 49 bp, Artificial Sequence
  Synthetic nucleotide
  misc_feature (29)..(29): h is a, c, or t
  misc_feature (30)..(30): n is a, c, g, or t
  misc_feature (31)..(31): h is a, c, or t
  misc_feature (32)..(32): n is a, c, g, or t
  misc_feature (33)..(33): h is a, c, or t
  misc_feature (34)..(34): n is a, c, g, or t
  misc_feature (35)..(35): h is a, c, or t
  misc_feature (36)..(36): n is a, c, g, or t
acacgacgctcttccgatcttgcatacghnhnhnhncagacagacttgt

SEQ ID NO: 90 - DNA, 49 bp, Artificial Sequence
  Synthetic nucleotide
  misc_feature (29)..(29): h is a, c, or t
  misc_feature (30)..(30): n is a, c, g, or t
  misc_feature (31)..(31): h is a, c, or t
  misc_feature (32)..(32): n is a, c, g, or t
  misc_feature (33)..(33): h is a, c, or t
  misc_feature (34)..(34): n is a, c, g, or t
  misc_feature (35)..(35): h is a, c, or t
  misc_feature (36)..(36): n is a, c, g, or t
acacgacgctcttccgatcttgcgcgtghnhnhnhncagacagacttgt

SEQ ID NO: 91 - DNA, 49 bp, Artificial Sequence
  Synthetic nucleotide
  misc_feature (29)..(29): h is a, c, or t
  misc_feature (30)..(30): n is a, c, g, or t
  misc_feature (31)..(31): h is a, c, or t
  misc_feature (32)..(32): n is a, c, g, or t
  misc_feature (33)..(33): h is a, c, or t
  misc_feature (34)..(34): n is a, c, g, or t
  misc_feature (35)..(35): h is a, c, or t
  misc_feature (36)..(36): n is a, c, g, or t
acacgacgctcttccgatcttgctacaghnhnhnhncagacagacttgt

SEQ ID NO: 92 - DNA, 49 bp, Artificial Sequence
  Synthetic nucleotide
  misc_feature (29)..(29): h is a, c, or t
  misc_feature (30)..(30): n is a, c, g, or t
  misc_feature (31)..(31): h is a, c, or t
  misc_feature (32)..(32): n is a, c, g, or t
  misc_feature (33)..(33): h is a, c, or t
  misc_feature (34)..(34): n is a, c, g, or t
  misc_feature (35)..(35): h is a, c, or t
  misc_feature (36)..(36): n is a, c, g, or t
acacgacgctcttccgatcttgtacgcahnhnhnhncagacagacttgt

SEQ ID NO: 93 - DNA, 49 bp, Artificial Sequence
  Synthetic nucleotide
  misc_feature (29)..(29): h is a, c, or t
  misc_feature (30)..(30): n is a, c, g, or t
  misc_feature (31)..(31): h is a, c, or t
  misc_feature (32)..(32): n is a, c, g, or t
  misc_feature (33)..(33): h is a, c, or t
  misc_feature (34)..(34): n is a, c, g, or t
  misc_feature (35)..(35): h is a, c, or t
  misc_feature (36)..(36): n is a, c, g, or t
acacgacgctcttccgatctttacggtghnhnhnhncagacagacttgt

SEQ ID NO: 94 - DNA, 49 bp, Artificial Sequence
  Synthetic nucleotide
  misc_feature (29)..(29): h is a, c, or t
  misc_feature (30)..(30): n is a, c, g, or t
  misc_feature (31)..(31): h is a, c, or t
  misc_feature (32)..(32): n is a, c, g, or t
  misc_feature (33)..(33): h is a, c, or t
  misc_feature (34)..(34): n is a, c, g, or t
  misc_feature (35)..(35): h is a, c, or t
  misc_feature (36)..(36): n is a, c, g, or t
acacgacgctcttccgatctttagccaghnhnhnhncagacagacttgt

SEQ ID NO: 95 - DNA, 49 bp, Artificial Sequence
  Synthetic nucleotide
  misc_feature (29)..(29): h is a, c, or t
  misc_feature (30)..(30): n is a, c, g, or t
  misc_feature (31)..(31): h is a, c, or t
  misc_feature (32)..(32): n is a, c, g, or t
  misc_feature (33)..(33): h is a, c, or t
  misc_feature (34)..(34): n is a, c, g, or t
  misc_feature (35)..(35): h is a, c, or t
  misc_feature (36)..(36): n is a, c, g, or t
acacgacgctcttccgatctttgaccgahnhnhnhncagacagacttgt

SEQ ID NO: 96 - DNA, 49 bp, Artificial Sequence
  Synthetic nucleotide
  misc_feature (29)..(29): h is a, c, or t
  misc_feature (30)..(30): n is a, c, g, or t
  misc_feature (31)..(31): h is a, c, or t
  misc_feature (32)..(32): n is a, c, g, or t
  misc_feature (33)..(33): h is a, c, or t
  misc_feature (34)..(34): n is a, c, g, or t
  misc_feature (35)..(35): h is a, c, or t
  misc_feature (36)..(36): n is a, c, g, or t
acacgacgctcttccgatctttgtggcahnhnhnhncagacagacttgt

SEQ ID NO: 97 - DNA, 20 bp, Artificial Sequence
  Anchor sequence
acacgacgctcttccgatct